European Patent Application EP 4 647 511 A1, published November 12, 2025. Title: GENE MARKER COMBINATION, KIT, AND DETECTION METHOD. Applicant: BEIJING XIANGXIN BIOTECHNOLOGY CO., LTD. Application EP. The sequence listing filed with the application follows.

SEQUENCE LISTING (56 sequences)

SEQ ID NO: 1 - DNA, 31 bp, synthetic construct
  misc_feature 1..31: note = ONECUT2-F1
  misc_feature 10: note = n = c or t
  misc_feature 19: note = n = c or t
  misc_feature 28: note = n = c or t
  source 1..31: mol_type = other DNA
gtttttgtgngtatatatngttatttgngtt

SEQ ID NO: 2 - DNA, 23 bp, synthetic construct
  misc_feature 1..23: note = ONECUT2-R1
  misc_feature 2: note = n = a or g
  misc_feature 13: note = n = a or g
  misc_feature 15: note = n = a or g
  source 1..23: mol_type = other DNA
cncattaacttcncnaacccaac

SEQ ID NO: 3 - DNA, 20 bp, synthetic construct
  misc_feature 1..20: note = ONECUT2-P1
  source 1..20: mol_type = other DNA
ttcggcgattcgtttgggcg

SEQ ID NO: 4 - DNA, 29 bp, synthetic construct
  misc_feature 1..29: note = ONECUT2-F2
  misc_feature 18: note = n = c or t
  source 1..29: mol_type = other DNA
tggtagtaagtttttagnggttagtttga

SEQ ID NO: 5 - DNA, 34 bp, synthetic construct
  misc_feature 1..34: note = ONECUT2-R2
  misc_feature 16: note = n = a or g
  source 1..34: mol_type = other DNA
tcaaataacccaaacnacatcataataaattaac

SEQ ID NO: 6 - DNA, 16 bp, synthetic construct
  misc_feature 1..16: note = ONECUT2-P2
  source 1..16: mol_type = other DNA
taggcggtcgagggtt

SEQ ID NO: 7 - DNA, 25 bp, synthetic construct
  misc_feature 1..25: note = ONECUT2-F3
  misc_feature 3: note = n = c or t
  misc_feature 5: note = n = c or t
  misc_feature 22: note = n = c or t
  source 1..25: mol_type = other DNA
ggngngttttttttagtagagngtt

SEQ ID NO: 8 - DNA, 25 bp, synthetic construct
  misc_feature 1..25: note = ONECUT2-R3
  misc_feature 10: note = n = a or g
  misc_feature 15: note = n = a or g
  misc_feature 21: note = n = a or g
  source 1..25: mol_type = other DNA
aaaactaacnaaacnacaccnctaa

SEQ ID NO: 9 - DNA, 22 bp, synthetic construct
  misc_feature 1..22: note = ONECUT2-P3
  source 1..22: mol_type = other DNA
agcgttacggtttcgcggtttt

SEQ ID NO: 10 - DNA, 32 bp, synthetic construct
  misc_feature 1..32: note = ONECUT2-F4
  misc_feature 6: note = n = c or t
  misc_feature 24: note = n = c or t
  source 1..32: mol_type = other DNA
gttaanggtagagtttaattagtngtagattt

SEQ ID NO: 11 - DNA, 29 bp, synthetic construct
  misc_feature 1..29: note = ONECUT2-R4
  misc_feature 8: note = n = a or g
  misc_feature 23: note = n = a or g
  source 1..29: mol_type = other DNA
aaaccacntttaattatccaacnaataca

SEQ ID NO: 12 - DNA, 23 bp, synthetic construct
  misc_feature 1..23: note = ONECUT2-P4
  source 1..23: mol_type = other DNA
ttacgcgtagattttttacgtag

SEQ ID NO: 13 - DNA, 31 bp, synthetic construct
  misc_feature 1..31: note = VIM-1-F1
  misc_feature 5: note = n = c or t
  misc_feature 13: note = n = c or t
  misc_feature 24: note = n = c or t
  source 1..31: mol_type = other DNA
ggttngtgttttngtttttttatngtaggat

SEQ ID NO: 14 - DNA, 29 bp, synthetic construct
  misc_feature 1..29: note = VIM-1-R1
  misc_feature 3: note = n = a or g
  misc_feature 11: note = n = a or g
  misc_feature 19: note = n = a or g
  source 1..29: mol_type = other DNA
acntaatcacntaactccnactaaaactc

SEQ ID NO: 15 - DNA, 20 bp, synthetic construct
  misc_feature 1..20: note = VIM-1-P1
  source 1..20: mol_type = other DNA
ttcggcggttcgggtatcgc

SEQ ID NO: 16 - DNA, 30 bp, synthetic construct
  misc_feature 1..30: note = VIM-1-F2
  misc_feature 6: note = n = c or t
  misc_feature 10: note = n = c or t
  misc_feature 21: note = n = c or t
  source 1..30: mol_type = other DNA
gttttngttngtttttttttngggagttag

SEQ ID NO: 17 - DNA, 30 bp, synthetic construct
  misc_feature 1..30: note = VIM-1-R2
  misc_feature 2: note = n = a or g
  misc_feature 10: note = n = a or g
  source 1..30: mol_type = other DNA
cnaaaacacnaacctaataaacataactac

SEQ ID NO: 18 - DNA, 27 bp, synthetic construct
  misc_feature 1..27: note = VIM-1-P2
  source 1..27: mol_type = other DNA
ttcgcgttatcgtcgtcgtttaggtta

SEQ ID NO: 19 - DNA, 36 bp, synthetic construct
  misc_feature 1..36: note = VIM-2-F1
  source 1..36: mol_type = other DNA
tttttagtattttagggtgagtttagtttagattat

SEQ ID NO: 20 - DNA, 30 bp, synthetic construct
  misc_feature 1..30: note = VIM-2-R1
  source 1..30: mol_type = other DNA
cctaaaactaaacataatcccgttacttca

SEQ ID NO: 21 - DNA, 26 bp, synthetic construct
  misc_feature 1..26: note = VIM-2-P1
  source 1..26: mol_type = other DNA
attcggaaagtttttaaaagttttag

SEQ ID NO: 22 - DNA, 22 bp, synthetic construct
  misc_feature 1..22: note = VIM-3-F1
  source 1..22: mol_type = other DNA
gagggagcgagataaagggatg

SEQ ID NO: 23 - DNA, 24 bp, synthetic construct
  misc_feature 1..24: note = VIM-3-R1
  misc_feature 4: note = n = a or g
  misc_feature 11: note = n = a or g
  source 1..24: mol_type = other DNA
cacnataaccncacaaacctacaa

SEQ ID NO: 24 - DNA, 17 bp, synthetic construct
  misc_feature 1..17: note = VIM-3-P1
  source 1..17: mol_type = other DNA
ttcgggggcggggatgg

SEQ ID NO: 25 - DNA, 30 bp, synthetic construct
  misc_feature 1..30: note = VIM-4-F1
  misc_feature 4: note = n = c or t
  misc_feature 15: note = n = c or t
  misc_feature 23: note = n = c or t
  source 1..30: mol_type = other DNA
ggtngagttttagtnggagttangtgatta

SEQ ID NO: 26 - DNA, 27 bp, synthetic construct
  misc_feature 1..27: note = VIM-4-R1
  misc_feature 4: note = n = a or g
  misc_feature 15: note = n = a or g
  misc_feature 17: note = n = a or g
  source 1..27: mol_type = other DNA
cacnacaaaaaaacncntaacatacac

SEQ ID NO: 27 - DNA, 22 bp, synthetic construct
  misc_feature 1..22: note = VIM-4-P1
  source 1..22: mol_type = other DNA
ttacgtttcgttttcgggcggc

SEQ ID NO: 28 - DNA, 17 bp, synthetic construct
  misc_feature 1..17: note = TERT-M2-F
  source 1..17: mol_type = other DNA
gctgggagggccaggaa

SEQ ID NO: 29 - DNA, 16 bp, synthetic construct
  misc_feature 1..16: note = TERT-M1-F
  source 1..16: mol_type = other DNA
gggccggggaccctga

SEQ ID NO: 30 - DNA, 18 bp, synthetic construct
  misc_feature 1..18: note = TERT-R
  source 1..18: mol_type = other DNA
ctcccagtggattcgcgg

SEQ ID NO: 31 - DNA, 19 bp, synthetic construct
  misc_feature 1..19: note = TERT-P
  source 1..19: mol_type = other DNA
ccacgtgggaagcgcggtc

SEQ ID NO: 32 - DNA, 18 bp, synthetic construct
  misc_feature 1..18: note = FGFR3-M1-F
  source 1..18: mol_type = other DNA
catctgcccccacagggt

SEQ ID NO: 33 - DNA, 17 bp, synthetic construct
  misc_feature 1..17: note = FGFR3-M2-F
  source 1..17: mol_type = other DNA
gcccccacagagcggtg

SEQ ID NO: 34 - DNA, 20 bp, synthetic construct
  misc_feature 1..20: note = FGFR3-R
  source 1..20: mol_type = other DNA
ttcacctccacgtgcttgag

SEQ ID NO: 35 - DNA, 21 bp, synthetic construct
  misc_feature 1..21: note = FGFR3-P
  source 1..21: mol_type = other DNA
tgggcagcgacgtggagttcc

SEQ ID NO: 36 - DNA, 30 bp, synthetic construct
  misc_feature 1..30: note = ONECUT2-F2
  source 1..30: mol_type = other DNA
atttttgtattattcgtttttgtgcgtata

SEQ ID NO: 37 - DNA, 28 bp, synthetic construct
  misc_feature 1..28: note = ONECUT2-R2
  source 1..28: mol_type = other DNA
gcgttttcggcgattcgtttgggcggtt

SEQ ID NO: 38 - DNA, 24 bp, synthetic construct
  misc_feature 1..24: note = ONECUT2-P2
  source 1..24: mol_type = other DNA
ccgttcaacgcattaacttcgcga

SEQ ID NO: 39 - DNA, 20 bp, synthetic construct
  misc_feature 1..20: note = ACTB-F
  source 1..20: mol_type = other DNA
ggttgtgtttagttaatggg

SEQ ID NO: 40 - DNA, 20 bp, synthetic construct
  misc_feature 1..20: note = ACTB-R
  source 1..20: mol_type = other DNA
aatcatctttcccaccaaac

SEQ ID NO: 41 - DNA, 23 bp, synthetic construct
  misc_feature 1..23: note = ACTB-P
  source 1..23: mol_type = other DNA
tataacctctacaaccttcaaaa

SEQ ID NO: 42 - DNA, 20 bp, synthetic construct
  misc_feature 1..20: note = ACTB-M1-M2-F
  source 1..20: mol_type = other DNA
gtcaggcagctcgtagctct

SEQ ID NO: 43 - DNA, 21 bp, synthetic construct
  misc_feature 1..21: note = ACTB-M1-M2-R
  source 1..21: mol_type = other DNA
atcgtgcgtgacattaaggag

SEQ ID NO: 44 - DNA, 24 bp, synthetic construct
  misc_feature 1..24: note = ACTB-M1-M2-P
  source 1..24: mol_type = other DNA
ccgtggccatctcttgctcgaagt

SEQ ID NO: 45 - DNA, 30 bp, synthetic construct
  misc_feature 1..30: note = EOMES-F1
  source 1..30: mol_type = other DNA
gttttttcgttgcgtttttttagatagatt

SEQ ID NO: 46 - DNA, 19 bp, synthetic construct
  misc_feature 1..19: note = EOMES-R1
  misc_feature 5: note = n = a or g
  misc_feature 14: note = n = a or g
  source 1..19: mol_type = other DNA
aaacntaccccccncttcc

SEQ ID NO: 47 - DNA, 29 bp, synthetic construct
  misc_feature 1..29: note = EOMES-P1
  source 1..29: mol_type = other DNA
aagagcggggtcgttatattttatcgttt

SEQ ID NO: 48 - DNA, 25 bp, synthetic construct
  misc_feature 1..25: note = TP53-F2
  source 1..25: mol_type = other DNA
ctttcttgcggagattctcttcctc

SEQ ID NO: 49 - DNA, 20 bp, synthetic construct
  misc_feature 1..20: note = TP53-R3
  source 1..20: mol_type = other DNA
aatgggacaggtaggacctg

SEQ ID NO: 50 - DNA, 22 bp, synthetic construct
  misc_feature 1..22: note = TP53-P1
  source 1..22: mol_type = other DNA
ctctcccaggacaggcacaaac

SEQ ID NO: 51 - DNA, 23 bp, synthetic construct
  misc_feature 1..23: note = TWIST1-F1
  misc_feature 6: note = n = c or t
  misc_feature 12: note = n = c or t
  source 1..23: mol_type = other DNA
ggaaanggtgtnggtgttgtaga

SEQ ID NO: 52 - DNA, 31 bp, synthetic construct
  misc_feature 1..31: note = TWIST1-R1
  misc_feature 6: note = n = a or g
  source 1..31: mol_type = other DNA
tacacnaaaatataaaaacctccaaatctac

SEQ ID NO: 53 - DNA, 22 bp, synthetic construct
  misc_feature 1..22: note = TWIST1-P1
  source 1..22: mol_type = other DNA
ttcgcgaggtgtttgggagttg

SEQ ID NO: 54 - DNA, 28 bp, synthetic construct
  misc_feature 1..28: note = PLEKHS1-593-F10
  source 1..28: mol_type = other DNA
tgatctagaagcttttttgcaattaaat

SEQ ID NO: 55 - DNA, 28 bp, synthetic construct
  misc_feature 1..28: note = PLEKHS1-90-93-R1
  source 1..28: mol_type = other DNA
tgaatacagtataccaagaggtcagtcc

SEQ ID NO: 56 - DNA, 23 bp, synthetic construct
  misc_feature 1..23: note = PLEKHS1-90-93-P1
  source 1..23: mol_type = other DNA
tgctgtatttctgttatgggcac